European Patent Application EP 4 324 473 A2, published February 21, 2024. Title: MULTIPARAMETRIC NUCLEIC ACID OPTIMIZATION. Applicant: ModernaTX, Inc. The sequence listing filed with the application follows.

SEQUENCE LISTING (3 sequences)

SEQ ID NO: 1 - protein, 267 aa, Homo sapiens
  source 1..267: note = Apolipoprotein A1 preproprotein
MKAAVLTLAVLFLTGSQARHFWQQDEPPQSPFDRVKDLATVYVDVLKDSGRDYVSQFEGSALGKQLNLKLLDNFDSVTSTFSKLREQLGPVTQEFFDNLEKETEGLRQEMSKDLEEVKAKVQPYLDDFQKKFQEEMELYRQKVEPLRAELQEGARQKLHELQEKLSPLGEEMRDRARAHVDALRTHLAPYSDELRQCLAARLEALKENGGARLAEYHAKATEHLSTLSEKAKPALEDLRQGLLPVLESFKVSFLSALEEYTKKLNTQ

SEQ ID NO: 2 - protein, 30 aa, Photinus pyralis
  source 1..30: note = N-terminal fragment from luciferin-4 monooxygenase (luciferase)
MEDAKNIKKGPAPFYPLEDGTAGEQLHKAM

SEQ ID NO: 3 - protein, 5 aa, synthetic construct
  source 1..5: note = Synthetic sequence
ADGSR